European Patent Application EP 4 796 640 A1, published August 26, 2026. Title: PLANTA ENRIQUECIDA EN AMINOÁCIDOS, PROTEÍNAS Y ALMIDÓN. Applicant: Universitat de València. The sequence listing filed with the application follows.

SEQUENCE LISTING (19 sequences)

SEQ ID NO: 1 - protein, 603 aa, synthetic construct [sequence omitted]

SEQ ID NO: 2 - protein, 288 aa, synthetic construct
  source 1..288: note = Amino acids 61 to 348 of Arabidopsis thaliana PGDH1 protein; note (original language) = Aminoácidos 61 a 348 de la proteína PGDH1 de Arabidopsis thaliana
KPTILVAEKLGDAGIKLLEDVANVDCSYNMTPEELNIKISLCDALIVRSGTKVGREVFESSHGRLKVVGRAGVGIDNVDLSAATEFGCLVVNAPTANTIAAAEHGIALMAAMARNVAQADASVKAGEWKRNKYVGVSLVGKTLAVLGFGKVGTEVARRAKGLGMRVIAHDPYAPADRAHAIGVDLVSFDEALATADFISLHMPLTPTTSKILNDETFAKMKKGVRIVNVARGGVIDEDALVRALDAGIVAQAALDVFTKEPPAKDSKLVQHERVTVTPHLGASTMEAQ

SEQ ID NO: 3 - protein, 14 aa, synthetic construct
  source 1..14: note = Amino acids 127 to 140 of Arabidopsis thaliana PGDH1 protein; note (original language) = Aminoácidos 127 a 140 de la proteína PGDH1 de Arabidopsis thaliana
VVGRAGVGIDNVDL

SEQ ID NO: 4 - protein, 12 aa, synthetic construct
  source 1..12: note = Amino acids 147 to 158 of Arabidopsis thaliana PGDH1 protein; note (original language) = Aminoácidos 147 a 158 de la proteína PGDH1 de Arabidopsis thaliana
GCLVVNAPTANT

SEQ ID NO: 5 - protein, 13 aa, synthetic construct
  source 1..13: note = Amino acids 192 to 204 of Arabidopsis thaliana PGDH1 protein; note (original language) = Aminoácidos 192 a 204 de la proteína PGDH1 de Arabidopsis thaliana
KYVGVSLVGKTLA

SEQ ID NO: 6 - protein, 11 aa, synthetic construct
  source 1..11: note = Amino acids 423 to 433 of Arabidopsis thaliana PGDH1 protein; note (original language) = Aminoácidos 423 a 433 de la proteína PGDH1 de Arabidopsis thaliana
DDLDTRLLRAM

SEQ ID NO: 7 - protein, 13 aa, synthetic construct
  source 1..13: note = Amino acids 532 to 544 of Arabidopsis thaliana PGDH1 protein; note (original language) = Aminoácidos 532 a 544 de la proteína PGDH1 de Arabidopsis thaliana
ILCRQVDQPGMIG

SEQ ID NO: 8 - DNA, 2227 bp, synthetic construct
  source 1..2227: mol_type = other DNA; note = Arabidopsis thaliana PGDH1 gene cDNA; note (original language) = ADNc del gen PGDH1 de Arabidopsis thaliana
cctgagccgactataaaaccttttagatctctccctcgtgttataactccgccaccaacaatatttttctctactcaattcactcacactccaaaagcggtagcaatgtcagccaccgccgccgcctcctcctcgatcgccgttgccaccaactctctcaggaacgtgactctgtcttccagatcgccccttccatcagccatctccgtggctttcccttcccgtggacgcaatactcttcagcgacgcctcgttctcgtttcctgcagtactggagacggatctaagcctacgattctcgtggcggagaagctcggtgacgctggtattaagcttttggaggatgtcgcgaatgtcgactgttcgtataacatgactcctgaggagctcaacattaagatctcgctctgtgacgccttgatcgtgaggagtgggactaaggttggccgtgaggtgttcgaatcgtctcacggacggctcaaggttgttggtcgcgctggtgttgggatcgacaacgtggatctgagtgcagcgacggagtttgggtgtttggttgtcaacgctccgacggcgaacacgatcgctgccgctgagcacggaatcgctcttatggccgccatggctaggaacgtagctcaagctgatgcgtctgttaaggctggagagtggaagaggaacaagtatgtaggtgtttcacttgtgggaaagacccttgcagtgttgggattcgggaaagttgggacggaagttgctcgtcgtgctaagggtcttggtatgcgtgtcattgctcatgatccctatgccccagcagaccgtgcacacgccattggtgttgacttagtgagctttgatgaagcccttgccaccgcggatttcatttctcttcatatgcctcttacgccaacaacatcgaagatactaaacgacgaaacctttgccaaaatgaagaagggagttcgaattgttaatgttgctcgtggaggtgtcatagacgaagatgcgttagtgagagctctggatgctggtattgttgcgcaggctgcacttgatgttttcaccaaagagcctccggctaaagatagcaagctcgtgcagcacgagagggtcactgtgacacctcatcttggagctagtaccatggaggctcaggaaggagttgccatcgaaattgctgaagctgttgttggagctctgaatggagagcttgctgctactgcagtcaatgcacctatggtttctgctgaggttctgaccgagctgaaaccatatgtggtgctagccgagaaactaggaagactggcagtgcaactggtggccggaggaagcggtgtgaaaaacgcgaaaatcacatacgcctcagcaagagccactgatgatcttgacaccagacttctccgagccatgatcaccaagggaatcatcgagccaatctctgacgtatatgtcaatttggtcaacgctgatttcacagccaagcagagaggtctcagactctcagaggaacgtgtgcttttggatggttcaccagagagcccattggagacaataactgttcagctaagcaatgtggagtccaaattcgccagttccctgtctgaatcaggagaggttaaagtggaaggaaaggttaaagacggagtcccgcatttgacaaaggttggatcttttgaggtcgatgtaactcttgaaggtagtatcatactgtgcaggcaggtggatcaacctggtatgatcgggactgtcggaagcatccttggagagtctaatgtcaatgttaacttcatgagcgttgggagaattgcaccgaggaagcaagcgattatggcgattggagtagatgacataccaagcaaagagacactgaagaagattggggaaattccagcggttgaggagttcgttttcctcaagctctagtttggtgtgttgttgattcttgaatcttaaatctcaccggtgaagatttgatgttgtttgttggtttaggcaataatgttattttggctttcatacagttttggtaacgttgagagtagtgtctctttgatgtttcaactttatggtttctattacttgagtgcttctttcttctctgaatatttatttcctgaatattagtgaccacaaattggtttataacccaattgaacgaaccgatgtaactatcgtagagaatctgttaattaagccaatccaatttttcaaaattggtttggtttggttcaga

SEQ ID NO: 9 - DNA, 2936 bp, synthetic construct
  source 1..2936: mol_type = other DNA; note = Arabidopsis thaliana PGDH1 gene; note (original language) = Gen PGDH1 de Arabidopsis thaliana
cctgagccgactataaaaccttttagatctctccctcgtgttataactccgccaccaacaatatttttctctactcaattcactcacactccaaaagcggtagcaatgtcagccaccgccgccgcctcctcctcgatcgccgttgccaccaactctctcaggaacgtgactctgtcttccagatcgccccttccatcagccatctccgtggctttcccttcccgtggacgcaatactcttcagcgacgcctcgttctcgtttcctgcagtactggagacggatctaagcctacgattctcgtggcggagaagctcggtgacgctggtattaagcttttggaggatgtcgcgaatgtcgactgttcgtataacatgactcctgaggagctcaacattaagatctcgctctgtgacgccttgatcgtgaggagtgggactaaggttggccgtgaggtgttcgaatcgtctcacggacggctcaaggttgttggtcgcgctggtgttgggatcgacaacgtggatctgagtgcagcgacggagtttgggtgtttggttgtcaacgctccgacggcgaacacgatcgctgccgctgagcacggaatcgctcttatggccgccatggctaggaacgtagctcaagctgatgcgtctgttaaggctggttagttcctttttgattcattgcctcaatttcatactttccatatgttgcgaaatatttattgattatgttctttctatacctgtgattgatggcttgttgtgtttattaatttgtatcatgagctttccttttcctgtactgttgttgacgatggtgaaatttaggatcgttacatttgctgattcttttgaaattgagttttgatcattcttgtctgttatctagctgacttgtggatcttggttttaataataccattgtaatgcaggagagtggaagaggaacaagtatgtaggtgtttcacttgtgggaaagacccttgcagtgttgggattcgggaaagttgggacggaagttgctcgtcgtgctaagggtcttggtatgcgtgtcattgctcatgatccctatgccccagcagaccgtgcacacgccattggtgttgacttagtgagctttgatgaagcccttgccaccgcggatttcatttctcttcatatgcctcttacgccaacaacatcgaagatactaaacgacgaaacctttgccaaaatgaagaagggagttcgaattgttaatgttgctcgtggaggtgtcatagacgaagatgcgttagtgagagctctggatgctggtattgttgcgcaggctgcacttgatgttttcaccaaagagcctccggctaaagatagcaagctcgtgcagcacgagagggtcactgtgacacctcatcttggagctagtaccatggaggctcaggtgtgcaattcattttacagttcaggtgataattaatcatgaaatttctgtttggcttctgttatatagttggtgttttggctttgacaggaaggagttgccatcgaaattgctgaagctgttgttggagctctgaatggagagcttgctgctactgcagtcaatgcacctatggtttctgctgaggtgagcactcgcttgtgctagtaaatacacacatattggtgttgtttcaaagaggcaaacttatcagcctatttactgtagctagcctgggaatgaatgtagcaaattatatttgttccgagttggttagaaagaagttagtgagcggcaaaattgttgaagtgagggtgggttttctagggatttgttttaagagcctcattaatcaagtttctgtgatttctgaattggattttagactagcaaggtttatagctttgttcttatcagattcaagttggaagatttcaattgttaagactatccatgtttgttatttgctcaagcttacatgcattctatctgcaggttctgaccgagctgaaaccatatgtggtgctagccgagaaactaggaagactggcagtgcaactggtggccggaggaagcggtgtgaaaaacgcgaaaatcacatacgcctcagcaagagccactgatgatcttgacaccagacttctccgagccatgatcaccaagggaatcatcgagccaatctctgacgtatatgtcaatttggtcaacgctgatttcacagccaagcagagaggtctcagactctcagaggaacgtgtgcttttggatggttcaccagagagcccattggagacaataactgttcagctaagcaatgtggagtccaaattcgccagttccctgtctgaatcaggagaggttaaagtggaaggaaaggttaaagacggagtcccgcatttgacaaaggttggatcttttgaggtcgatgtaactcttgaaggtagtatcatactgtgcaggcaggtggatcaacctggtatgatcgggactgtcggaagcatccttggagagtctaatgtcaatgttaacttcatgagcgttgggagaattgcaccgaggaagcaagcgattatggcgattggagtagatgacataccaagcaaagagacactgaagaagattggggaaattccagcggttgaggagttcgttttcctcaagctctagtttggtgtgttgttgattcttgaatcttaaatctcaccggtgaagatttgatgttgtttgttggtttaggcaataatgttattttggctttcatacagttttggtaacgttgagagtagtgtctctttgatgtttcaactttatggtttctattacttgagtgcttctttcttctctgaatatttatttcctgaatattagtgaccacaaattggtttataacccaattgaacgaaccgatgtaactatcgtagagaatctgttaattaagccaatccaatttttcaaaattggtttggtttggttcaga

SEQ ID NO: 10 - DNA, 18 bp, synthetic construct
  source 1..18: mol_type = other DNA; note = PSAT1+1 For primer; note (original language) = Cebador PSAT1+1 For
atggcggctacgacgaac

SEQ ID NO: 11 - DNA, 21 bp, synthetic construct
  source 1..21: mol_type = other DNA; note = PSAT1+1270 Rev primer; note (original language) = Cebador PSAT1+1270 Rev
agcatgcttagcctggaaatc

SEQ ID NO: 12 - DNA, 20 bp, synthetic construct
  source 1..20: mol_type = other DNA; note = 2x35S -786 For primer; note (original language) = Cebador 2x35S -786 For
ggtcactgtcacaacgtcgc

SEQ ID NO: 13 - DNA, 29 bp, synthetic construct
  source 1..29: mol_type = other DNA; note = T-Nos +322 BglII Rev primer; note (original language) = Cebador T-Nos +322 BglII Rev
ggaagatctccggctcgtatgttgtgtgg

SEQ ID NO: 14 - DNA, 33 bp, synthetic construct
  source 1..33: mol_type = other DNA; note = EDA9GFP XbaI AvrII For primer; note (original language) = Cebador EDA9GFP XbaI AvrII For
tgcctaggctctagagcccttatgtcagccacc

SEQ ID NO: 15 - DNA, 31 bp, synthetic construct
  source 1..31: mol_type = other DNA; note = EDA9GFP SpeI Rev primer; note (original language) = Cebador EDA9GFP SpeI Rev
gactagtggggaaattcgagctcttagtggt

SEQ ID NO: 16 - protein, 28 aa, synthetic construct
  source 1..28: note = Amino acids 203 to 230 of Arabidopsis thaliana PGDH1 protein; note (original language) = Aminoácidos 203 a 230 de la proteína PGDH1 de Arabidopsis thaliana
LAVLGFGKVGTEVARRAKGLGMRVIAHD

SEQ ID NO: 17 - protein, 23 aa, synthetic construct
  source 1..23: note = Amino acids 251 to 273 of Arabidopsis thaliana PGDH1 protein; note (original language) = Aminoácidos 251 a 273 de la proteína PGDH1 de Arabidopsis thaliana
ALATADFISLHMPLTPTTSKILN

SEQ ID NO: 18 - protein, 17 aa, synthetic construct
  source 1..17: note = Amino acids 280 to 296 of Arabidopsis thaliana PGDH1 protein; note (original language) = Aminoácidos 280 a 296 de la proteína PGDH1 de Arabidopsis thaliana
MKKGVRIVNVARGGVID

SEQ ID NO: 19 - protein, 73 aa, synthetic construct
  source 1..73: note = Amino acids 530 to 603 of Arabidopsis thaliana PGDH1 protein; note (original language) = Aminoácidos 530 a 603 de la proteína PGDH1 de Arabidopsis thaliana
IILCRQVDQPGMIGTVGSILGESNVNVNFMSVGRIAPRKQAIMAIGVDDIPSKETLKKIGEIPAVEEFVFLKL